European Patent Application EP 4 502 184 A1, published February 5, 2025. Title: Methods for testing for late recurrence of ER-positive breast cancer and screening for therapeutic agents. Applicant: Japanese Foundation for Cancer Research. The sequence listing filed with the application follows.

SEQUENCE LISTING (41 sequences)

SEQ ID NO: 1 - DNA, 16 bp, synthetic construct
  misc_feature 1..16: note = ELEANOR2-LNA
  source 1..16: mol_type = other DNA
tttggccacattggaa

SEQ ID NO: 2 - DNA, 15 bp, synthetic construct
  misc_feature 1..15: note = LNA-Control
  source 1..15: mol_type = other DNA
aacacgtctatacgc

SEQ ID NO: 3 - DNA, 20 bp, synthetic construct
  misc_feature 1..20: note = PCR primer
  source 1..20: mol_type = other DNA
ctcctcctcatcctctccca

SEQ ID NO: 4 - DNA, 20 bp, synthetic construct
  misc_feature 1..20: note = PCR primer
  source 1..20: mol_type = other DNA
ctttggtccgtctcctccac

SEQ ID NO: 5 - DNA, 20 bp, synthetic construct
  misc_feature 1..20: note = PCR primer
  source 1..20: mol_type = other DNA
taagccaatgtcagggcaag

SEQ ID NO: 6 - DNA, 21 bp, synthetic construct
  misc_feature 1..21: note = PCR primer
  source 1..21: mol_type = other DNA
tcccgagctcatatgcattac

SEQ ID NO: 7 - DNA, 19 bp, synthetic construct
  misc_feature 1..19: note = PCR primer
  source 1..19: mol_type = other DNA
cgcctctgaagtttgcatc

SEQ ID NO: 8 - DNA, 19 bp, synthetic construct
  misc_feature 1..19: note = PCR primer
  source 1..19: mol_type = other DNA
gtctgggtgccactgtttg

SEQ ID NO: 9 - DNA, 20 bp, synthetic construct
  misc_feature 1..20: note = PCR primer
  source 1..20: mol_type = other DNA
cccagatggagaaagctctg

SEQ ID NO: 10 - DNA, 20 bp, synthetic construct
  misc_feature 1..20: note = PCR primer
  source 1..20: mol_type = other DNA
gttgtttgctgcacagatgg

SEQ ID NO: 11 - DNA, 23 bp, synthetic construct
  misc_feature 1..23: note = PCR primer
  source 1..23: mol_type = other DNA
ttcagaaggttgtgtggcgtaga

SEQ ID NO: 12 - DNA, 20 bp, synthetic construct
  misc_feature 1..20: note = PCR primer
  source 1..20: mol_type = other DNA
cagcttctgttggcacctta

SEQ ID NO: 13 - DNA, 19 bp, synthetic construct
  misc_feature 1..19: note = PCR primer
  source 1..19: mol_type = other DNA
ccattgctgagttagctgc

SEQ ID NO: 14 - DNA, 20 bp, synthetic construct
  misc_feature 1..20: note = PCR primer
  source 1..20: mol_type = other DNA
aaacggcttagatgaaggag

SEQ ID NO: 15 - DNA, 23 bp, synthetic construct
  misc_feature 1..23: note = PCR primer
  source 1..23: mol_type = other DNA
gtttcactgtgttgggcacacta

SEQ ID NO: 16 - DNA, 20 bp, synthetic construct
  misc_feature 1..20: note = PCR primer
  source 1..20: mol_type = other DNA
attttaaaacgagccaggca

SEQ ID NO: 17 - DNA, 20 bp, synthetic construct
  misc_feature 1..20: note = PCR preimer
  source 1..20: mol_type = other DNA
tagtagaggctgttcccttc

SEQ ID NO: 18 - DNA, 20 bp, synthetic construct
  misc_feature 1..20: note = PCR primer
  source 1..20: mol_type = other DNA
ctgtaaccttacccatagcc

SEQ ID NO: 19 - DNA, 20 bp, synthetic construct
  misc_feature 1..20: note = PCR primer
  source 1..20: mol_type = other DNA
tcatgagcaatgcgtggctt

SEQ ID NO: 20 - DNA, 20 bp, synthetic construct
  misc_feature 1..20: note = PCR primer
  source 1..20: mol_type = other DNA
caaggcttggttctaagcag

SEQ ID NO: 21 - DNA, 22 bp, synthetic construct
  misc_feature 1..22: note = PCR primer
  source 1..22: mol_type = other DNA
aagaatgtctgatggtgccctg

SEQ ID NO: 22 - DNA, 21 bp, synthetic construct
  misc_feature 1..21: note = PCR primer
  source 1..21: mol_type = other DNA
caagtagaactccagagtgag

SEQ ID NO: 23 - DNA, 20 bp, synthetic construct
  misc_feature 1..20: note = PCR primer
  source 1..20: mol_type = other DNA
gaagtctcttctcgaatgct

SEQ ID NO: 24 - DNA, 20 bp, synthetic construct
  misc_feature 1..20: note = PCR primer
  source 1..20: mol_type = other DNA
tctcaagtcccgtatcttca

SEQ ID NO: 25 - DNA, 20 bp, synthetic construct
  misc_feature 1..20: note = PCR primer
  source 1..20: mol_type = other DNA
gaatgaacaagactcctgac

SEQ ID NO: 26 - DNA, 20 bp, synthetic construct
  misc_feature 1..20: note = PCR primer
  source 1..20: mol_type = other DNA
tctggcgcaggtaagttgta

SEQ ID NO: 27 - DNA, 20 bp, synthetic construct
  misc_feature 1..20: note = PCR primer
  source 1..20: mol_type = other DNA
ctagcacttcatgtgattct

SEQ ID NO: 28 - DNA, 20 bp, synthetic construct
  misc_feature 1..20: note = PCR primer
  source 1..20: mol_type = other DNA
ccattgtacagcactgttct

SEQ ID NO: 29 - DNA, 22 bp, synthetic construct
  misc_feature 1..22: note = PCR primer
  source 1..22: mol_type = other DNA
tttgaagcacccctctcttcct

SEQ ID NO: 30 - DNA, 20 bp, synthetic construct
  misc_feature 1..20: note = PCR primer
  source 1..20: mol_type = other DNA
gtccttagtacctcgttcct

SEQ ID NO: 31 - DNA, 20 bp, synthetic construct
  misc_feature 1..20: note = PCR primer
  source 1..20: mol_type = other DNA
gctccccagagagaaattaa

SEQ ID NO: 32 - DNA, 20 bp, synthetic construct
  misc_feature 1..20: note = PCR primer
  source 1..20: mol_type = other DNA
gcctatcactacagaagaca

SEQ ID NO: 33 - DNA, 20 bp, synthetic construct
  misc_feature 1..20: note = PCR primer
  source 1..20: mol_type = other DNA
agcaacggcagatgagtatc

SEQ ID NO: 34 - DNA, 20 bp, synthetic construct
  misc_feature 1..20: note = PCR primer
  source 1..20: mol_type = other DNA
ccaggatcaccttcttttgc

SEQ ID NO: 35 - DNA, 20 bp, synthetic construct
  misc_feature 1..20: note = PCR primer
  source 1..20: mol_type = other DNA
ccgtggttgttggtagaatg

SEQ ID NO: 36 - DNA, 20 bp, synthetic construct
  misc_feature 1..20: note = PCR primer
  source 1..20: mol_type = other DNA
aatcgattggtggactctgg

SEQ ID NO: 37 - DNA, 19 bp, synthetic construct
  misc_feature 1..19: note = PCR primer
  source 1..19: mol_type = other DNA
agcgcccgaggaaacttac

SEQ ID NO: 38 - DNA, 20 bp, synthetic construct
  misc_feature 1..20: note = PCR primer
  source 1..20: mol_type = other DNA
agcattttgagccacattcc

SEQ ID NO: 39 - DNA, 21 bp, synthetic construct
  misc_feature 1..21: note = PCR primer
  source 1..21: mol_type = other DNA
caggccaaattcagataatcg

SEQ ID NO: 40 - DNA, 20 bp, synthetic construct
  misc_feature 1..20: note = PCR primer
  source 1..20: mol_type = other DNA
tccttggcagattccatagc

SEQ ID NO: 41 - DNA, 16 bp, synthetic construct
  misc_feature 1..16: note = pa-ELEANOR-LNA
  source 1..16: mol_type = other DNA
gtgccagactccgata